European Patent Application EP 4 279 923 A1, published November 22, 2023. Title: METHOD AND KIT FOR DETERMINING THE DEGREE OF BACTERIAL CONTAMINATION OF FOOD AND BEVERAGE SAMPLE OR ENVIRONMENTAL SAMPLE. Applicant: ASAHI KASEI KABUSHIKI KAISHA. The sequence listing filed with the application follows.

SEQUENCE LISTING (14 sequences)

SEQ ID NO: 1 - protein, 118 aa, Artificial Sequence
  PA51B2 VH
QVQLQQPGSVLVRPGASVKLSCKPSGYTFTGSWMHWTKQRPGQGLEWIGEIHPYSGNTNYNEKFRVKATLTVDTSSSTTYVDLSSLTSDDSAVYYCASGDFDAGFTYWGQGTLVTVSA

SEQ ID NO: 2 - protein, 111 aa, Artificial Sequence
  PA51B2 VL
DIVLTQSPASLAVSLGRRATISCKASQSVDYDGDSYMNWYQQKPGQPPKLLIYVASNLESGIPARFSGSGSGTDFTLNIHPVEEEDAATYYCQQTNEDPFTFGAGTKLELK

SEQ ID NO: 3 - protein, 120 aa, Artificial Sequence
  LP54A3 VH
EVQLQQSGAELVKPGASVRLSCSASGFNIKDTYMHWMRQRPEQGLEWIGRIDPANGNAKYDPKFQVKATITADTSSNTASLQFSSLTSEDTAVYFCASESLDDMYYFDYWGQGTTLTVSS

SEQ ID NO: 4 - protein, 107 aa, Artificial Sequence
  LP54A3 VL
DIVMTQSQKFMSTSVGDRVSVTCKASQNVGVNVAWYQQKPGQSPKALIYSASYRYSGVPDRFTGSGSGTDFTLTISNVQSEDLAEYFCQQYHSYLYTFGGGTKLEIK

SEQ ID NO: 5 - protein, 118 aa, Artificial Sequence
  CP141A190.1 VH
QVQLQQPGAELVKPGASVKLSCKTSGYNFTSNWIHWVKQRPGQGLEWIGEINPSNGRANYNEKFKNKATLTVDKSSSTAFMHLSSLTSEDSAVYFCSRGDFDEGFTYWGQGTLVTVSA

SEQ ID NO: 6 - protein, 108 aa, Artificial Sequence
  CP141A190.1 VL
QIVLTQSPAIMSASLGERVTMTCTASSNVNSDYLHWYQQKPGSSPRLWIYTTSNLASGVPTRFSGNGSGTSYSLTISSMEAEDAATYYCHQYHRSPRTFGGGTKLEIK

SEQ ID NO: 7 - protein, 120 aa, Artificial Sequence
  HI142D11.3 VH
EVQLQQSGAELVKPGASVKLSCTASGFNIKDTYIHWVKQRPEQGLEWIGRIDPANGNTKYDPKFQGKATITADTSSNTAYLQLSSLTSEDTAVYYCPRPYGYVGWYFDVWGAGTTVTVSS

SEQ ID NO: 8 - protein, 107 aa, Artificial Sequence
  HI142D11.3 VL
DIVMTQSHKFMSTSVGDRVSITCKASQDVRNAVAWYQQKPGQSPKLLISSASYRYSGVPDRFTGSGSGTDFTFTISSVQAEDLAVYYCQQHYDTPPTFGGGTKLEIK

SEQ ID NO: 9 - protein, 115 aa, Artificial Sequence
  SA75B2 VH
EVLLQQSGPELVKPGASVKIPCKASGYTFTDYHMDWVKQSHGKSLEWIGEINPNNGGTIYNQKFKGKATLTVDKSSSTAYMELRSLTSEDTAVYYCARSGVFTYWGQGTLVTVSA

SEQ ID NO: 10 - protein, 112 aa, Artificial Sequence
  SA75B2 VL
DVVMTQTPLSLPVSLGDQASISCRSSQSLVYSNGNTYLHWYLQKPGQSPKLLIYKVSNRFSGVPDRFSGSGSGTDFTLKISRVEAEDLGVYFCSQSTHVPLTFGAGTKLELK

SEQ ID NO: 11 - protein, 114 aa, Artificial Sequence
  PA78A2 VH
EVQLQQSGAEFLNPGASVKLSCTASGFTIIDIYIHWVKQRPEQGLEWIGRIDSANGKTKYDPKFQGKATITSDTSSNTAYLQLSSLTSEDTAVYYCARYSSGYWGQGTLVTVSA

SEQ ID NO: 12 - protein, 106 aa, Artificial Sequence
  PA78A2 VL
DIQMTQSPSSLSASLGGKVTITCKASQDINKYIAWYQHKPGKGPRLLIHYTSTLQPGIPSRFSGSGSGRDYSFSISNLEPEDIATYYCLQYDILWTFGGGTKLEIK

SEQ ID NO: 13 - protein, 116 aa, Artificial Sequence
  EC50C1 VH
QVQLQQSGAELAKPGASVKMSCKASGYTFTSYWMNWVKQRPGQGLEWIGYINPNTGYTEYDQKFKDKATLTADKSSSTAYMQLSSLTSEDSAVYYCARYWAYFEYWGQGTTLTVSS

SEQ ID NO: 14 - protein, 106 aa, Artificial Sequence
  EC50C1 VL
DIKMTQSPSSMYASLGERVTITCKASQDINSYLSWFQQKPGKSPKTLIYRANRLVDGVPSRFSGSGSGQDYSLTISSLEYEDMGIYYCLQYDEFRTFGGGTKLEIK